European Patent Specification EP 3 601 552 B1, published July 1, 2026. Title: POLYPEPTIDES HAVING DNASE ACTIVITY. Applicant: Novozymes A/S. The sequence listing filed with the application follows.

SEQUENCE LISTING (48 sequences)

SEQ ID NO: 1 - DNA, 751 bp, Ascobolus stictoideus
  CDS (1)..(242)
  sig_peptide (1)..(54)
  mat_peptide (55)..(748)
  CDS (310)..(572)
  CDS (639)..(748)
atgaagctcactttcctcaccgctcttgctgcctctttggctctcaccgctgccaacccactcccagctccagctccaccaaacatcccatccgctgccaccgcaaagtctgagcttgctgctctcggcaccagaaccagcgatgcccctggttactcccgcgatctcttcaaccactggatcaccatttctggccaatgcaacacccgcgagactgtcctcaagcgtgacggaaccaacgtgtaagaccaccctcctcctcctcctacattgttgcaaacataaatactaacaaaaagccctctatagtgtccaagcctccaactgcgctgccacctccggaacctggtactctcccttcgatggcgccacctggaccgccgcctccgacctcgacattgaccacgttgtcccactctccaacgcctggaagtctggagccggaacttggactgctgctcgtcgtcaacagttcgcaaatgacttggttaacccccaactcattgccgttactgattcggtcaaccaggccaagggtgataagtcccctgatgcctggaagccaccacttagtaagttcttcccccatgatccatccacatgaaaggattgaattgagataccaacctttgatatagcctcttactactgcacctacgccaggatgtgggttagagtcaagtatgtttacggcttgactgtcactgctgctgagaagtcggctttgactagcatgttgaacacttgctag

SEQ ID NO: 2 - protein, 205 aa, Ascobolus stictoideus
MKLTFLTALAASLALTAANPLPAPAPPNIPSAATAKSELAALGTRTSDAPGYSRDLFNHWITISGQCNTRETVLKRDGTNVVQASNCAATSGTWYSPFDGATWTAASDLDIDHVVPLSNAWKSGAGTWTAARRQQFANDLVNPQLIAVTDSVNQAKGDKSPDAWKPPLTSYYCTYARMWVRVKYVYGLTVTAAEKSALTSMLNTC

SEQ ID NO: 3 - protein, 187 aa, Ascobolus stictoideus
NPLPAPAPPNIPSAATAKSELAALGTRTSDAPGYSRDLFNHWITISGQCNTRETVLKRDGTNVVQASNCAATSGTWYSPFDGATWTAASDLDIDHVVPLSNAWKSGAGTWTAARRQQFANDLVNPQLIAVTDSVNQAKGDKSPDAWKPPLTSYYCTYARMWVRVKYVYGLTVTAAEKSALTSMLNTC

SEQ ID NO: 4 - DNA, 973 bp, Urnula sp-56769
  CDS (1)..(227)
  sig_peptide (1)..(48)
  mat_peptide (49)..(970)
  CDS (310)..(433)
  CDS (493)..(549)
  CDS (614)..(670)
  CDS (741)..(804)
  CDS (861)..(970)
atgaagttttccaccgttcttcctctcgtgttcactctggtcgcgggggcaccagcgccaacaccgatcgtcgaccaagctgcaatcgagaagcgtctgccaacaggcattcccaccgccgctaccgcaaagaccttgttggctgggttgggcaccagaactactgatgcgactggatacgaccgggacctgttcccgcactggatcaccatttctggaaactgcaagtgcgttttgaacccagccttagattatctaccaaatcagtatttcttgtgtatcaatcattctaagacgtatggattacagcacccgtgagacggtcttaaaccgtgacggcacgaaccttgatattggcaccgattgttaccctgacagcggcacctgggtcagtccttatgatggagctacctggactgcggcttcggatgtggtatgtttccaacaacttaatacgcatagaattcacatactaatactccatttaactaggatatcgaccatgttgtgccgctgtctgaagcttggaaagctggtgcgaatgcatgggtacttagcacaatatctctactcacacaattagctcatactaatacacttcatcttcctgaagactactgcccagcgccaggcattcgccaatgacctcaccaatcctcaattagtcgctgtgagtttctttcccttcacagacaggtaaacaacctggaaactcagggatgctgattgaacgtgttcaggtcacggataatgtcaactccgccaagggtgataagacccccgacctttggaagcccccgttgagtatgttttcctcttgtacgacatgcttggaatcttactaaccacgtttataacagcctcgttccactgcacctatgcccggatgtacgtcaaggtcaagagcgtctacagcctcacggttaagtctgctgagaggacggcccttacttctatgttggctacttgttaa

SEQ ID NO: 5 - protein, 213 aa, Urnula sp-56769
MKFSTVLPLVFTLVAGAPAPTPIVDQAAIEKRLPTGIPTAATAKTLLAGLGTRTTDATGYDRDLFPHWITISGNCNTRETVLNRDGTNLDIGTDCYPDSGTWVSPYDGATWTAASDVDIDHVVPLSEAWKAGANAWTTAQRQAFANDLTNPQLVAVTDNVNSAKGDKTPDLWKPPLTSFHCTYARMYVKVKSVYSLTVKSAERTALTSMLATC

SEQ ID NO: 6 - protein, 197 aa, Urnula sp-56769
APAPTPIVDQAAIEKRLPTGIPTAATAKTLLAGLGTRTTDATGYDRDLFPHWITISGNCNTRETVLNRDGTNLDIGTDCYPDSGTWVSPYDGATWTAASDVDIDHVVPLSEAWKAGANAWTTAQRQAFANDLTNPQLVAVTDNVNSAKGDKTPDLWKPPLTSFHCTYARMYVKVKSVYSLTVKSAERTALTSMLATC

SEQ ID NO: 7 - DNA, 728 bp, Ascobolus sp. ZY179
  CDS (1)..(242)
  sig_peptide (1)..(54)
  mat_peptide (55)..(725)
  CDS (294)..(556)
  CDS (616)..(725)
atgaaggtcactttcctcgccgctctcgctgccactttggctctcacttctgccaatccgctcccagtcccaactccaccaaacattccatccgctaccaccgcgaaggctgagttggctgccctcggcaccagaaccaccgacgccaccggctactctcgtgactacttcaaccattggatcaccatctcgggcgcgtgcaacactcgtgagactgttctcaagcgtgatggaaccaacgtgtaagctctacttttgcgttatatgcatccatgctgacaaagagactatagtgttaccgactctagctgctatgccacctccggaacctggtactctccatttgacggtgccacctggaccgccgcctccgatgtcgatatcgaccacgtcgttcctctctccaacgcctggaagtctggtgccaacacctggacttcttccagacgccagcaattcgccaatgacttgaccaaccctcaactcattgccgtcacagacgacgtcaaccaagccaagggtgacaagtctccagatgcctggaagccaccacttagtaagttcaatctcaaacacttgaaagtcattgaatcggacgactaacttgtttttcagcctcctactactgcacctacgccaagatgtgggttcgtgtcaagtatgtctacgacttgactgtcaccgccgctgagaagagcgctttgaccagcatgttgaacacttgctaa

SEQ ID NO: 8 - protein, 205 aa, Ascobolus sp. ZY179
MKVTFLAALAATLALTSANPLPVPTPPNIPSATTAKAELAALGTRTTDATGYSRDYFNHWITISGACNTRETVLKRDGTNVVTDSSCYATSGTWYSPFDGATWTAASDVDIDHVVPLSNAWKSGANTWTSSRRQQFANDLTNPQLIAVTDDVNQAKGDKSPDAWKPPLTSYYCTYAKMWVRVKYVYDLTVTAAEKSALTSMLNTC

SEQ ID NO: 9 - protein, 187 aa, Ascobolus sp. ZY179
NPLPVPTPPNIPSATTAKAELAALGTRTTDATGYSRDYFNHWITISGACNTRETVLKRDGTNVVTDSSCYATSGTWYSPFDGATWTAASDVDIDHVVPLSNAWKSGANTWTSSRRQQFANDLTNPQLIAVTDDVNQAKGDKSPDAWKPPLTSYYCTYAKMWVRVKYVYDLTVTAAEKSALTSMLNTC

SEQ ID NO: 10 - DNA, 907 bp, Morchella costata
  CDS (1)..(197)
  sig_peptide (1)..(45)
  mat_peptide (46)..(904)
  CDS (248)..(371)
  CDS (492)..(605)
  CDS (662)..(725)
  CDS (795)..(904)
atgaagctcacagcagtagccctcttctttacgaccgctctcgcagctcctacgctagagaagcgaactcctcctaatattcccactgccgcttccgcgaatactatgcttgccgctctcacaacaaggaccacagatgccactggttactcccgcgatcttttcccgcattggattacccagagcgggtcttgcaagtaaggcatctggtaatcattcataaatttcattcctgacgaaagagcagcacccgtgaggtagttcttgcccgcgatggatccaacgtggtccaggccagcgactgctcagcctcgagcggaacctggttttcgccttacgacggtgcgacctggaccgctgcttctgatcttgtaagttttcattgccacatgtggcttgatatttgcatgagatgctcgccgggagaaaaaaacccgtcgatatttttttatttttttggcggtaggcactgacatatccgactgtttcaggacattgatcatgttgtgcctctctccgatgcatggaagtccggggccaacacctggactacagccggacgtcaagcctttgccaacgatctcacgaacccccagttgattgccgtaagtcgttaattctctgctgcctcgagggaacataaactgacggcgtggttcaggtcaccgataatgtaaatcaggccaagggtgataagtcgcctgatgcgtggaaaccacctctcagtaagttcttttgtttttccatcagtttttttcagcgaaaagagaactaaccctaatatctgtgttcagcatcgtactactgcacctatgcaaggatgtgggttaaggtgaagagtgtgtattcattgtctgtgacctcagctgagcgttcggcgttgacgagcatgttgaacacgtgctga

SEQ ID NO: 11 - protein, 203 aa, Morchella costata
MKLTAVALFFTTALAAPTLEKRTPPNIPTAASANTMLAALTTRTTDATGYSRDLFPHWITQSGSCNTREVVLARDGSNVVQASDCSASSGTWFSPYDGATWTAASDLDIDHVVPLSDAWKSGANTWTTAGRQAFANDLTNPQLIAVTDNVNQAKGDKSPDAWKPPLTSYYCTYARMWVKVKSVYSLSVTSAERSALTSMLNTC

SEQ ID NO: 12 - protein, 188 aa, Morchella costata
APTLEKRTPPNIPTAASANTMLAALTTRTTDATGYSRDLFPHWITQSGSCNTREVVLARDGSNVVQASDCSASSGTWFSPYDGATWTAASDLDIDHVVPLSDAWKSGANTWTTAGRQAFANDLTNPQLIAVTDNVNQAKGDKSPDAWKPPLTSYYCTYARMWVKVKSVYSLSVTSAERSALTSMLNTC

SEQ ID NO: 13 - DNA, 822 bp, Trichobolus zukalii
  CDS (1)..(175)
  sig_peptide (1)..(57)
  mat_peptide (58)..(819)
  CDS (234)..(402)
  CDS (464)..(642)
  CDS (710)..(819)
atgcatttctcatccttcgtcctcccggtgattgcgctggcatccagcgctctggctgctccgactccggctcccctcctcgagaagcgttctcctccgaatatcccatccaagtcttccgcggtctcaatgcttgcaggcctcagcacacgaaccagcgatgccaccggatatggtatgttccagcattcaaagggagataggctgcattcgaaaactgacaatatctacagaccgcgatctcttcccccactggatcacaatctctggcacctgcaatacccgtgagaccgtcctcaagcgcgacgccagttccatcactgttggcgacaactgtgccgctacctctggatcgtggttttcgccgtacgatggcgccacctggacggctgcttccgacctgtaagcatgcatttttttttttttttaccctcctgtgaacgttcctctaacagcttcccagtgatatcgaccatgttgttcctttgagtgacgcctggaagtctggtgccaatacctggaccaccgccaagcgccaaacctttgccaatgatctgaccaacccccagcttattgctgttaccgataatgtcaaccaggctaagggagataagtccccggacgcatggaagccgcccttgtgtaagtttcccgagtctccgttctgtgtatccccttcgaggagattgatgctaatggattcttacagcctcttactactgcacctacgccaagatgtgggtcaaggtcaaaagcgcttatgggctttccgtcaaggctgctgagaggactgctttgacttccatgttgaacacttgctag

SEQ ID NO: 14 - protein, 211 aa, Trichobolus zukalii
MHFSSFVLPVIALASSALAAPTPAPLLEKRSPPNIPSKSSAVSMLAGLSTRTSDATGYDRDLFPHWITISGTCNTRETVLKRDASSITVGDNCAATSGSWFSPYDGATWTAASDLDIDHVVPLSDAWKSGANTWTTAKRQTFANDLTNPQLIAVTDNVNQAKGDKSPDAWKPPLSSYYCTYAKMWVKVKSAYGLSVKAAERTALTSMLNTC

SEQ ID NO: 15 - protein, 192 aa, Trichobolus zukalii
APTPAPLLEKRSPPNIPSKSSAVSMLAGLSTRTSDATGYDRDLFPHWITISGTCNTRETVLKRDASSITVGDNCAATSGSWFSPYDGATWTAASDLDIDHVVPLSDAWKSGANTWTTAKRQTFANDLTNPQLIAVTDNVNQAKGDKSPDAWKPPLSSYYCTYAKMWVKVKSAYGLSVKAAERTALTSMLNTC

SEQ ID NO: 16 - DNA, 787 bp, Trichophaea saccata
  CDS (1)..(158)
  sig_peptide (1)..(51)
  mat_peptide (52)..(784)
  CDS (215)..(437)
  CDS (493)..(592)
  CDS (654)..(784)
atgaagttctctcctcttgccctcctcggcctcgtcgccagcgcctctgcggctgcgatcgagaagcgcacgccaccaaacattcccagcacttccagcgccaagtccatgcttgcgggtttgagcgttcggaccactgatgccactggttacgaccggttagtgaacccactgccacgcacgtgatgtcggtcgttaatggtcactcctccagatccctcttccctcactggatcactatctctggcacgtgcgacactcgtgagacggtgctgaaccgtgatggcaccggcctcactatcggcagtgactgctaccctactgccggcacctggtactctccatacgacggagccacctggactgcagcctcggatttggacatcgaccacgttgtccccctttctgacgcatggaagtcgggtgcaaatctctgggtacattccctccccctcttttccttcagtgggcaataactaacatcatgaacagactacctcccagcgccagaacttcgccaatgaccttaccaacccgcagctgattgcggttacggataacgtcaaccaggcaaagggtgacaagagccctggtatatagccccacccgaaccagtatcctctcactgtaccgacggctgacttgagaaaaagatttgtggaagcccccgttgacttcgtaccattgcacatatgccaagatgtgggttaaggtcaagagcgtgtactccctctcggtcaccgccgctgagaagtcggccttgacgtccatgttgaacacctgttaa

SEQ ID NO: 17 - protein, 204 aa, Trichophaea saccata
MKFSPLALLGLVASASAAAIEKRTPPNIPSTSSAKSMLAGLSVRTTDATGYDRSLFPHWITISGTCDTRETVLNRDGTGLTIGSDCYPTAGTWYSPYDGATWTAASDLDIDHVVPLSDAWKSGANLWTTSQRQNFANDLTNPQLIAVTDNVNQAKGDKSPDLWKPPLTSYHCTYAKMWVKVKSVYSLSVTAAEKSALTSMLNTC

SEQ ID NO: 18 - protein, 187 aa, Trichophaea saccata
AAIEKRTPPNIPSTSSAKSMLAGLSVRTTDATGYDRSLFPHWITISGTCDTRETVLNRDGTGLTIGSDCYPTAGTWYSPYDGATWTAASDLDIDHVVPLSDAWKSGANLWTTSQRQNFANDLTNPQLIAVTDNVNQAKGDKSPDLWKPPLTSYHCTYAKMWVKVKSVYSLSVTAAEKSALTSMLNTC

SEQ ID NO: 19 - DNA, 784 bp, Trichophaea minuta
  CDS (1)..(158)
  sig_peptide (1)..(51)
  mat_peptide (52)..(781)
  CDS (215)..(437)
  CDS (494)..(593)
  CDS (651)..(781)
atgaagttctctcctcttgccctttttggcctcgtcgccagcgtatctgccgctgcaatcgagaagcgcacacctccaaacattcccagcacctccagcgcccagtctatgctttcgggcttgagcattcggaccactaatgccactggttacgaccggttagtaaaccatcgttcacatacgagatatccagtgtttaacattccccatctagctctctcttccctcactggatcaccatctctggcaactgcgacacccgcgagacagtgctgaaccgtgacggaaccgaccttaccatcggcagcgactgctatcctagtgacggcacttggtactctccctacgacggcgccacttggactgccgcctcggatttggacatcgatcacgttgttcccctttccgatgcttggaagtcgggtgcaaacctctgggtatctccacactccgcccctcatgtctagaaggcaatatttaatgtcataatcagactactgcccagcgccagaacttcgcaaatgacctctccaacccgcagcttattgcggtcacggacagtgtcaaccaagcaaagagtgacaagagccctggtatgcctccaccaccatcctctcactgaaggcaaccccccgctgacataatgaaagatttgtggaagcccccgctcacctcgtaccactgcacttacgccaagatgtgggttaaggtcaagagtgtttactccctctcggtcacttcggctgagaagtcggctttgacgtctatgttgaacacgtgttaa

SEQ ID NO: 20 - protein, 204 aa, Trichophaea minuta
MKFSPLALFGLVASVSAAAIEKRTPPNIPSTSSAQSMLSGLSIRTTNATGYDRSLFPHWITISGNCDTRETVLNRDGTDLTIGSDCYPSDGTWYSPYDGATWTAASDLDIDHVVPLSDAWKSGANLWTTAQRQNFANDLSNPQLIAVTDSVNQAKSDKSPDLWKPPLTSYHCTYAKMWVKVKSVYSLSVTSAEKSALTSMLNTC

SEQ ID NO: 21 - protein, 187 aa, Trichophaea minuta
AAIEKRTPPNIPSTSSAQSMLSGLSIRTTNATGYDRSLFPHWITISGNCDTRETVLNRDGTDLTIGSDCYPSDGTWYSPYDGATWTAASDLDIDHVVPLSDAWKSGANLWTTAQRQNFANDLSNPQLIAVTDSVNQAKSDKSPDLWKPPLTSYHCTYAKMWVKVKSVYSLSVTSAEKSALTSMLNTC

SEQ ID NO: 22 - DNA, 787 bp, Trichophaea minuta
  CDS (1)..(158)
  sig_peptide (1)..(51)
  mat_peptide (52)..(784)
  CDS (215)..(437)
  CDS (494)..(593)
  CDS (654)..(784)
atgaagttctctcctcttgccctctttggcctcgtcgccagcgcctctgccgctgcaatcgagaagcgcactcccccaaacattcccagcacctccagcgccaagtccatgctttcgggcttgagcattcggaccactgatgccactggttacgaccggttagtaaaccatcattcacacacgagatatccagtgtttaacattccccacccagctctctcttcccccactggatcaccatctctggcaactgcgacacccgcgagacagtgctgaaccgtgacggaaccggccttaccatcggcagcgactgctaccctagtgccggcacttggtactctccctacgacggagccacctggactgccgcctcggatttggacatcgaccacgttgttcccctttccgatgcttggaagtcgggtgcaaacctctgggtatctccacactccacccctcatgtctagaaggcaatatttaacgtcatattcagactaccgcccagcgccagaacttcgcaaatgacctctccaacccgcagcttattgcggtcacggataatgtcaaccaagcaaagagtgacaagagccctggtatgcctccaccaccaccatcctctcactgaaggcaccccccgctgacataatgaaaagatttgtggaagcccccgctcacctcgtaccactgcacttacgccaagatgtgggttaaggtcaagagtgtttactccctctcggtcacttcggctgagaagtcggctttgacgtctatgttgaacacgtgttaa

SEQ ID NO: 23 - protein, 204 aa, Trichophaea minuta
MKFSPLALFGLVASASAAAIEKRTPPNIPSTSSAKSMLSGLSIRTTDATGYDRSLFPHWITISGNCDTRETVLNRDGTGLTIGSDCYPSAGTWYSPYDGATWTAASDLDIDHVVPLSDAWKSGANLWTTAQRQNFANDLSNPQLIAVTDNVNQAKSDKSPDLWKPPLTSYHCTYAKMWVKVKSVYSLSVTSAEKSALTSMLNTC

SEQ ID NO: 24 - protein, 187 aa, Trichophaea minuta
AAIEKRTPPNIPSTSSAKSMLSGLSIRTTDATGYDRSLFPHWITISGNCDTRETVLNRDGTGLTIGSDCYPSAGTWYSPYDGATWTAASDLDIDHVVPLSDAWKSGANLWTTAQRQNFANDLSNPQLIAVTDNVNQAKSDKSPDLWKPPLTSYHCTYAKMWVKVKSVYSLSVTSAEKSALTSMLNTC

SEQ ID NO: 25 - DNA, 793 bp, Trichophaea abundans
  CDS (1)..(158)
  sig_peptide (1)..(51)
  mat_peptide (52)..(790)
  CDS (215)..(437)
  CDS (502)..(601)
  CDS (660)..(790)
atgaagttctctcctcttgccttcttcggcctcgtcgccagcgtctcggccgctgcagtcgagaagcgtacacctccaaacattcccagcaccaccagcgccaagtccatgctttcaggcttgaacattcggactactgatgccactggttacgaccggttagtaaaccatcacatacaactaatattcgatagttaacagttcccccatccagcgccctcttcccccattggatcaccatctctggcaactgcaacacccgcgagacggtgctgaaccgtgacggaaccggcctcacgatcggtagcgactgctaccccagttccggcacctggttctctccctacgacggagccacctggactgcagcctcggatttggacatcgaccacgttgtacccctttccgatgcttggaagtcgggtgcaaatctctgggtatatatccgctttttttcttgtgtgatggcatcggaaattgttaatcaatgcctttaaaaagactaccgctcagcgccagaacttcgccaatgacctctctaacccgcagctaatcgcggtcacggacaatgtcaactctgcaaagggtgataagagccctggtacgcacctccctccctccctcctctcaatgattgctgctgacatcatgatcaaaagatttgtggaagcccccgctctcctcgtactactgcacttacgccaaaatgtgggttaaggtcaagagcgtgtactcgctgtcggtgacctctgctgagaagtcggctttgacgtctatgttgaacacgtgttaa

SEQ ID NO: 26 - protein, 204 aa, Trichophaea abundans
MKFSPLAFFGLVASVSAAAVEKRTPPNIPSTTSAKSMLSGLNIRTTDATGYDRALFPHWITISGNCNTRETVLNRDGTGLTIGSDCYPSSGTWFSPYDGATWTAASDLDIDHVVPLSDAWKSGANLWTTAQRQNFANDLSNPQLIAVTDNVNSAKGDKSPDLWKPPLSSYYCTYAKMWVKVKSVYSLSVTSAEKSALTSMLNTC

SEQ ID NO: 27 - protein, 187 aa, Trichophaea abundans
AAVEKRTPPNIPSTTSAKSMLSGLNIRTTDATGYDRALFPHWITISGNCNTRETVLNRDGTGLTIGSDCYPSSGTWFSPYDGATWTAASDLDIDHVVPLSDAWKSGANLWTTAQRQNFANDLSNPQLIAVTDNVNSAKGDKSPDLWKPPLSSYYCTYAKMWVKVKSVYSLSVTSAEKSALTSMLNTC

SEQ ID NO: 28 - DNA, 618 bp, Pseudoplectania nigrella
  sig_peptide (1)..(54)
  CDS (1)..(615)
  mat_peptide (55)..(615)
atgaagttctctgtttccaccattgtcttcggccttgttgccacttcctctgctgccgccattgaaaagcggactcctcccaacatcccctccgccagctccgcaaagaccatgcttgcatccatccccgtcagaaccactgatgcaactggataccaacgctcccttttcccccactggatcaccatctccggtcaatgcaacacccgtgaaaccgtcctcaaccgtgacggaaccaacctttccatcggcagcgattgctatcccgacagtggaacctggttctcagtttatgacggagccacctggacccaagcttctgaccttgacatcgaccatgttgtgccactttccgacgcctggaagtcaggtgccaatacttggaccactgccaagcgccaggactttgcaaacgacttgacaaacccccagttgattgcggttacggatactgttaaccaggcaaagggtgataagagcccggatgcttggaagcctcctcttactaactaccactgcacctacgctaaaatgtgggttaaggttaaaagtgtttggggactctcggtgacggctcccgaaaaaagtgctttgactagtatgttgaacacctgttga

SEQ ID NO: 29 - protein, 205 aa, Pseudoplectania nigrella
MKFSVSTIVFGLVATSSAAAIEKRTPPNIPSASSAKTMLASIPVRTTDATGYQRSLFPHWITISGQCNTRETVLNRDGTNLSIGSDCYPDSGTWFSVYDGATWTQASDLDIDHVVPLSDAWKSGANTWTTAKRQDFANDLTNPQLIAVTDTVNQAKGDKSPDAWKPPLTNYHCTYAKMWVKVKSVWGLSVTAPEKSALTSMLNTC

SEQ ID NO: 30 - protein, 187 aa, Pseudoplectania nigrella
AAIEKRTPPNIPSASSAKTMLASIPVRTTDATGYQRSLFPHWITISGQCNTRETVLNRDGTNLSIGSDCYPDSGTWFSVYDGATWTQASDLDIDHVVPLSDAWKSGANTWTTAKRQDFANDLTNPQLIAVTDTVNQAKGDKSPDAWKPPLTNYHCTYAKMWVKVKSVWGLSVTAPEKSALTSMLNTC

SEQ ID NO: 31 - DNA, 957 bp, Gyromitra esculenta
  CDS (1)..(197)
  sig (1)..(45)
  mat_peptide (46)..(954)
  CDS (255)..(378)
  CDS (448)..(504)
  CDS (585)..(641)
  CDS (703)..(766)
  CDS (845)..(954)
atgaagttctcaatctttgcgcttttcatctcagtcgccgctgccgctccagttttggagaagaggacaccgccgaatgtccctagcggagctactgccaaaaccctgcttacgtctctgtctgtcaggaccactgatgccactggatatgatcgtgaccttttcccacactggatcacccagagcggtacctgcaagtacgtcccccagtcggatcttttttttccgcccgagtgctgacggctctgctatagcacccgcgaggttgtcttgaagcgtgatggaactagtgttgtccaagcaagcgattgttcggccaccagcggatcatggttcagtccctacgatggtgctacctggacagctgcttccgatctcgtacgctacccacccccgaagaatcattcgtacgtatcgtatcagctaacactgggggaaaaaatccaggacattgaccatgttgtcccgctttctgacgcctggaagtctggcgcaaacgcctgggtaattcattcctcctcctcctactagtatatgtagcgcaggggggtaacgaactactgacaaaaaaaaaaaacgaaaagacaactgccaaacgccagtcctttgccaacgacctcacaaacccccaactaattgctgtgcgtcccccactctcatccctcgaaccctacaatggccctaagaactaaaggtccacaggttaccgataacgtcaaccaatccaaaggtgacaaatcacctgacctttggaagccacccctcggtaagttatatatcattgcaatgttagctacatacttgggaaatactaatgtttttcccgggggggggatgggggcagcttcatattactgcacatacgcatgtatgtgggttaaggtcaagagtgtctgggcgctttctgtcacagctgctgagaagtctgcgcttacgagcatgcttaatacgtgctag

SEQ ID NO: 32 - protein, 203 aa, Gyromitra esculenta
MKFSIFALFISVAAAAPVLEKRTPPNVPSGATAKTLLTSLSVRTTDATGYDRDLFPHWITQSGTCNTREVVLKRDGTSVVQASDCSATSGSWFSPYDGATWTAASDLDIDHVVPLSDAWKSGANAWTTAKRQSFANDLTNPQLIAVTDNVNQSKGDKSPDLWKPPLASYYCTYACMWVKVKSVWALSVTAAEKSALTSMLNTC

SEQ ID NO: 33 - protein, 188 aa, Gyromitra esculenta
APVLEKRTPPNVPSGATAKTLLTSLSVRTTDATGYDRDLFPHWITQSGTCNTREVVLKRDGTSVVQASDCSATSGSWFSPYDGATWTAASDLDIDHVVPLSDAWKSGANAWTTAKRQSFANDLTNPQLIAVTDNVNQSKGDKSPDLWKPPLASYYCTYACMWVKVKSVWALSVTAAEKSALTSMLNTC

SEQ ID NO: 34 - DNA, 904 bp, Morchella esculenta
  CDS (1)..(197)
  sig_peptide (1)..(45)
  mat_peptide (46)..(901)
  CDS (247)..(370)
  CDS (488)..(601)
  CDS (655)..(718)
  CDS (792)..(901)
atgaagctcacagcagtagtcctcttcttcacgaccgctctcgcagctcctacgctagagaagcggactcctcctaatattcctactgccgcttccgcgaagactatgcttgacgctctcacaacaaggaccacagatgccactggttactcccgtgatctcttcccgcattggattacccagagcgggtcttgcaagtaaggcatctggtaatcattcataagattcattcctgacaaagagtagtacccgtgaggtagttcttgcccgcgatggatccagcgtggtccaggccagtgactgctcagcctcgagcgggacctggttttccccttacgacggtgcgacctggaccgctgcatctgatcttgtaagttttcattacaacatgcagtttgagatttgcataagatgctcgccgggaaattaaagcccgtcgatatatttttgttttggcggtaggcactgacacatccggccatttcaggacattgatcatgttgtgcctctctctgatgcatggaagtccggggccgacacctggactacagccagacgtcaaacctttgccaacgatctcacgaatccccagttgatcgccgtaagtcaattctcccctacttcgagggaacataaactgatggtgtggttcaggtcaccgataatgtaaatcaggcgaagggtgataagtcgcctgatgcgtggaaaccgcctcttagtaagttttttccattcggctttttttttttttttttagctaaaagagaactaaccctaatatttgtgtccagcatcgtactactgcacttatgcaaggatgtgggttaaggtgaagagtgtgtattcgttgtctgtgacctcagctgagaagacggcattgacgagtatgttgaacacgtgctga

SEQ ID NO: 35 - protein, 203 aa, Morchella esculenta
MKLTAVVLFFTTALAAPTLEKRTPPNIPTAASAKTMLDALTTRTTDATGYSRDLFPHWITQSGSCNTREVVLARDGSSVVQASDCSASSGTWFSPYDGATWTAASDLDIDHVVPLSDAWKSGADTWTTARRQTFANDLTNPQLIAVTDNVNQAKGDKSPDAWKPPLTSYYCTYARMWVKVKSVYSLSVTSAEKTALTSMLNTC

SEQ ID NO: 36 - protein, 188 aa, Morchella esculenta
APTLEKRTPPNIPTAASAKTMLDALTTRTTDATGYSRDLFPHWITQSGSCNTREVVLARDGSSVVQASDCSASSGTWFSPYDGATWTAASDLDIDHVVPLSDAWKSGADTWTTARRQTFANDLTNPQLIAVTDNVNQAKGDKSPDAWKPPLTSYYCTYARMWVKVKSVYSLSVTSAEKTALTSMLNTC

SEQ ID NO: 37 - DNA, 905 bp, Morchella crassipes
  CDS (1)..(197)
  sig_peptide (1)..(45)
  mat_peptide (46)..(902)
  CDS (247)..(370)
  CDS (488)..(601)
  CDS (655)..(718)
  CDS (793)..(902)
atgaagctcacagcagtagtcctctttttcacgaccgctctcgcagctcctacgctagagaagcggactcctcccaatattcccactgccgcttccgcgaagactatgcttgacgctctcacaacaaggactacagatgctactggttactcccgtgatctcttcccgcattggattacccagagcgggtcttgcaagtaaggcatctggtaatcattcataaggttcattcctgacaaagagtagtacccgtgaggtagttcttgcccgcgatggatccagcgtggtccaggccagtgactgctcagcctcgagcgggacctggttttccccttacgacggtgcgacctggaccgctgcatctgatcttgtaagttttcattacaacatgcagtttgagatttgcataagatgctcgctgggaaattaaagctcgtcgatatatttttgttttggcggtaggcactgacacatccggccatttcaggacattgatcatgttgtgcctctctctgatgcatggaagtccggggccgacacctggactacagccaaacgtcaaacctttgccaacgatctcacgaatccccagttgatcgccgtaagtcaattctcccctacttcgagggaacataaactgatggtgtggttcaggtcaccgataatgtaaatcaggcgaagggtgataagtcgcctgatgcgtggaaaccgcctcttagtaagttttttttcattcggctttttttttttttttttagctaaaagagaaccaaccctaatatttgtgtccagcatcgtactactgcacttatgcaaggatgtgggttaaggtgaagagtgtgtattcgttgtctgtgacctcagctgagaagacggcattgacgagtatgttgaacacgtgctga

SEQ ID NO: 38 - protein, 203 aa, Morchella crassipes
MKLTAVVLFFTTALAAPTLEKRTPPNIPTAASAKTMLDALTTRTTDATGYSRDLFPHWITQSGSCNTREVVLARDGSSVVQASDCSASSGTWFSPYDGATWTAASDLDIDHVVPLSDAWKSGADTWTTAKRQTFANDLTNPQLIAVTDNVNQAKGDKSPDAWKPPLTSYYCTYARMWVKVKSVYSLSVTSAEKTALTSMLNTC

SEQ ID NO: 39 - protein, 188 aa, Morchella crassipes
APTLEKRTPPNIPTAASAKTMLDALTTRTTDATGYSRDLFPHWITQSGSCNTREVVLARDGSSVVQASDCSASSGTWFSPYDGATWTAASDLDIDHVVPLSDAWKSGADTWTTAKRQTFANDLTNPQLIAVTDNVNQAKGDKSPDAWKPPLTSYYCTYARMWVKVKSVYSLSVTSAEKTALTSMLNTC

SEQ ID NO: 40 - DNA, 841 bp, Disciotis venosa
  CDS (1)..(197)
  sig_peptide (1)..(45)
  mat_peptide (46)..(838)
  CDS (253)..(376)
  CDS (438)..(551)
  CDS (607)..(670)
  CDS (729)..(838)
atgaagctctctgctattgtcatttttatctcagccgttgctgctgctccagctttggagaagaggactcccccaaacattcccactgcggcatctgcaaagactttgcttgctgcattgaccactaggactactgatgccaccgggtatgatcgtgatcttttccctcactggattacccagagcggatcctgcaagtaagttaatggaacgcctaacacctccaactactctctaatatttccatcttagcacccgcgaggttgtcctggcacgcgatggaaccaatgtcgtccaggccagcgattgctctgcttcaagtgggacatggttctccccctacgatggtgctacatggactgctgcctcagatctcgtatgtaacccaattgagtaattgtgctagatatcgtattaacagtgccgcctgaatctaggacattgaccacgttgtcccactttcggatgcctggaagtctggtgcgggaacctggaccactgctaagcgtcaatcattcgccaacgaccttacaaacccccagctgattgctgtaagccacattatactccccaagttggtgcatcgactaagctgatatctctcaggttaccgacaacgtcaaccaagccaagggtgacaagtcccccgacgcctggaagccccctctcagtaagccgcctcatcacctgcctcttgggctgagtaaatactaacattagttttctagcctcatactactgcacctacgcccgtatgtgggtcaaggtcaagagtgtctgggaactctctgtcaccgcggctgagaggactgccctcacgagcatgctcaacacatgctag

SEQ ID NO: 41 - protein, 203 aa, Disciotis venosa
MKLSAIVIFISAVAAAPALEKRTPPNIPTAASAKTLLAALTTRTTDATGYDRDLFPHWITQSGSCNTREVVLARDGTNVVQASDCSASSGTWFSPYDGATWTAASDLDIDHVVPLSDAWKSGAGTWTTAKRQSFANDLTNPQLIAVTDNVNQAKGDKSPDAWKPPLTSYYCTYARMWVKVKSVWELSVTAAERTALTSMLNTC

SEQ ID NO: 42 - protein, 188 aa, Disciotis venosa
APALEKRTPPNIPTAASAKTLLAALTTRTTDATGYDRDLFPHWITQSGSCNTREVVLARDGTNVVQASDCSASSGTWFSPYDGATWTAASDLDIDHVVPLSDAWKSGAGTWTTAKRQSFANDLTNPQLIAVTDNVNQAKGDKSPDAWKPPLTSYYCTYARMWVKVKSVWELSVTAAERTALTSMLNTC

SEQ ID NO: 43 - protein, 5 aa, Artificial
  Motif
  MISC_FEATURE (1)..(1): X=E (Glu), D (Asp), H (His)
  MISC_FEATURE (3)..(3): X=I (Ile), V (Val), L (Leu), F (Phe), M (Met)
  misc_feature (4)..(4): Xaa can be any naturally occurring amino acid
  MISC_FEATURE (5)..(5): X=P (Pro), A (Ala), S (Ser)
XHXXX

SEQ ID NO: 44 - protein, 5 aa, Artificial
  Motif
  MISC_FEATURE (1)..(1): X= T (Tyr), D (Asp), S (Ser)
  MISC_FEATURE (2)..(2): X= G (Gly), N (Asn)
XXPQL

SEQ ID NO: 45 - protein, 5 aa, Artificial
  Motif
  MISC_FEATURE (1)..(1): X= F (Phe), L (Leu), Y (Tyr), I (Ile)
  MISC_FEATURE (3)..(3): X= N (Asn), R (Arg)
  MISC_FEATURE (5)..(5): X= L (leu), I (Ile), P (Pro), V (Val)
XAXDX

SEQ ID NO: 46 - protein, 4 aa, Artificial
  Motif
  MISC_FEATURE (2)..(2): X= Asp (D), Asn (N)
  MISC_FEATURE (4)..(4): X= A (Ala), R (Arg)
CXTX

SEQ ID NO: 47 - protein, 4 aa, Artificial
  Motif
  MISC_FEATURE (1)..(1): X= D (Asp), Q (Gln)
  MISC_FEATURE (2)..(2): X= I (Ile), V (Val)
XXDH

SEQ ID NO: 48 - protein, 8 aa, Artificial
  Motif
  MISC_FEATURE (3)..(3): X=T (Thr), S (Ser)
  MISC_FEATURE (4)..(4): X=D (Asp), N (Asn)
  MISC_FEATURE (5)..(5): X=A (Ala), P (Pro)
  MISC_FEATURE (6)..(6): X=T (Thr), D (Asp), P (Pro), S (Ser)
RTXXXXGY